European Patent Specification EP 3 709 021 B1, published March 19, 2025. Title: A method for predicting response to anti PD-1 antibody or anti PD-L1 antibody therapy , a method for evaluating cancer malignancy, and a method for increasing response to anti PD-1 antibody or anti PD-L1 antibody therapy. Applicant: J-Pharma Co., Ltd NATIONAL UNIVERSITY CORPORATION GUNMA UNIVERSITY OSAKA UNIVERSITY. The sequence listing filed with the application follows.

SEQUENCE LISTING (4 sequences)

SEQ ID NO: 1 - DNA, 21 bp, Artificial  Sequence
  siPD-L1#2 Sense
  misc_feature (1)..(19): RNA fragment
  misc_feature (20)..(21): DNA fragment
ggacucacuugguaauucutt

SEQ ID NO: 2 - DNA, 21 bp, Artificial  Sequence
  siPD-L1#2 Antisense
  misc_feature (1)..(19): RNA fragment
  misc_feature (20)..(21): DNA fragment
agaauuaccaagugagucctt

SEQ ID NO: 3 - DNA, 21 bp, Artificial  Sequence
  siLAT1#3 Sense
  misc_feature (1)..(19): RNA fragment
  misc_feature (20)..(21): DNA fragment
uguccaaucuagaucccaatt

SEQ ID NO: 4 - DNA, 21 bp, Artificial  Sequence
  siLAT1#3 Antisense
  misc_feature (1)..(19): RNA fragment
  misc_feature (20)..(21): DNA fragment
uugggaucuagauuggacaca